European Patent Specification EP 3 530 674 B1, published April 24, 2024. Title: Composite polypeptide monomer, associate of the composite polypeptide monomers having cell permeabilization, and norovirus component vaccine for subcutaneous, intradermal, transdermal or intramuscular administration containing the associate as active ingredient. Applicant: Denka Company Limited Tokyo Institute of Technology Japan as Represented by Director-General of National Institute of Infectious Diseases Katayama, Kazuhiko. The sequence listing filed with the application follows.

SEQUENCE LISTING (29 sequences)

SEQ ID NO: 1 - protein, 16 aa, Artificial Sequence
  repeating sequence
LEGSNTIFVRGDETKT

SEQ ID NO: 2 - protein, 86 aa, Bacteriophage T4
VEGNGTILVKGNVTIIVEGNADITVKGDATTLVEGNQTNTVNGNLSWKVAGTVDWDVGGDWTEKMASMSSISSGQYTIDGSRIDIG

SEQ ID NO: 3 - protein, 125 aa, Bacteriophage P2
VEGNGTILVKGNVTIIVEGNADITVKGDATTLDALHIRFPDGAVIEYEPETSALTVSGIKTASVTASGSVTATVPVVMVKASTRVTLDTPEVVCTNRLITGTLEVQKGGTMRGNIEHTGGELSSN

SEQ ID NO: 4 - protein, 107 aa, Bacteriophage Mu
VEGNGTILVKGNVTIIVEGNADITVKGDATTLGDAGIYHHEGHRIRLTKDGRCIITCKTVEVYADESMTVDTPRTTFTGDVEIQKGLGVKGKSQFDSNITAPDAIIN

SEQ ID NO: 5 - protein, 110 aa, Bacteriophage phi 92
VEGNGTILVKGNVTIIVEGNADITVKGDATTLEKVIISNNKQTYASFDPNGNISVYNTQGMKIDMTPNSIVLTDAGGGKLTLQGGTMTYKGGTVNLNGLTITPDGRMTDS

SEQ ID NO: 6 - protein, 27 aa, Bacteriophage T4
GYIPEAPRDGQAYVRKDGEWVLLSTFL

SEQ ID NO: 7 - protein, 21 aa, Bacteriophage P2
GKVLHTHKHPGDSGGTTGSPL

SEQ ID NO: 8 - protein, 23 aa, Bacteriophage Mu
GKSTDKHIHRGDSGGTTGPMQLE

SEQ ID NO: 9 - protein, 30 aa, Bacteriophage phi 92
GGIGLHTHTHPVRGVETGGSTVTSDKPNGG

SEQ ID NO: 10 - protein, 327 aa, Mouse norovirus
IERTIYRMVDLPVLQPRLCTHARWPAPIYGLLVDPSLPSNPQWQNGRVHVDGTLLGTTPVSGSWVSCFAAEAAYEFQSGIGEVATFTLIEQDGSAYVPGDRAAPLGYPDFSGQLEIEVQTETTKKGEKLKVTTFEMILGPTTNVDQVPYQGRVYASLTAAASLDLVDGRVRAVPRSVYGFQDVVPEYNDGLLVPLAPPIGPFLPGEVLLRFRTYMRQIDSTDAAAEAIDCALPQEFVSWFASNAFTVQSEALLLRYRNTLTGQLLFECKLYSEGYIALSYSGSGPLTFPTDGFFEVVSWVPRLYQLASVGSLATGRTLKQMDELYKE

SEQ ID NO: 11 - protein, 131 aa, Mouse norovirus
VSGSWVSCFAAEAAYEFQSGIGEVATFTLIEQDGSAYVPGDRAAPLGYPDFSGQLEIEVQTETTKKGEKLKVTTFEMILGPTTNVDQVPYQGRVYASLTAAASLDLVDGRVRAVPRSVYGFQDVMDELYKE

SEQ ID NO: 12 - protein, 322 aa, Human norovirus
PFTVPILTVEEMTNSRFPIPLEKLFTGPSGAFVVQPQNGRCTTDGVLLGTTQLSPVNICTFRGDVTHIAGSRNYTMNLASLNWNNYDPTEEIPAPLGTPDFVGKIQGLLTQTTKGDGSTRGHKATVYTGSAPFTPKLGSVQFSTDTENDFETHQNTKFTPVGVIQDGSTTHRNEPQQWVLPSYSGRNVHNVHLAPAVAPTFPGEQLLFFRSTMPGCSGYPNMDLDCLLPQEWVQHFYQEAAPAQSDVALLRFVNPDTGRVLFECKLHKSGYVTVAHTGQHDLVIPPNGYFRFDSWVNQFYTLAPMGNGTGRRRALMDELYKE

SEQ ID NO: 13 - protein, 135 aa, Human norovirus
LSPVNICTFRGDVTHIAGSRNYTMNLASLNWNNYDPTEEIPAPLGTPDFVGKIQGLLTQTTKGDGSTRGHKATVYTGSAPFTPKLGSVQFSTDTENDFETHQNTKFTPVGVIQDGSTTHRNEPQQWVLMDELYKE

SEQ ID NO: 14 - protein, 7 aa, Artificial Sequence
  a part of linker sequence in GFP
MDELYKE

SEQ ID NO: 15 - protein, 16 aa, Artificial Sequence
  linker sequence in GFP
MDELYKQSNSSSVPGG

SEQ ID NO: 16 - protein, 8 aa, Artificial Sequence
  modification sequence
VEHHHHHH

SEQ ID NO: 17 - protein, 232 aa, Artificial Sequence
  GFP (green fluorescent protein)
MSKGEELFTGVVPILVELDGDVNGHKFSVRGEGEGDATNGKLTLKFICTTGKLPVPWPTLVTTLTYGVQCFSRYPDHMKRHDFFKSAMPEGYVQERTISFKDDGTYKTRAEVKFEGDTLVNRIELKGIDFKEDGNILGHKLEYNFNSHNVYITADKQKNGIKANFKIRHNVEDGSVQLADHYQQNTPIGDGPVLLPDNHYLSTQSVLSKDPNEKRDHMVLLEFVTAAGITHG

SEQ ID NO: 18 - DNA, 20 bp, Artificial Sequence
  primer
ctgcagatggatgaactgta

SEQ ID NO: 19 - DNA, 20 bp, Artificial Sequence
  primer
catatgtatatctccttctt

SEQ ID NO: 20 - DNA, 35 bp, Artificial Sequence
  primer
ttcatccatctgcagtaaagcacgtctgcgccccg

SEQ ID NO: 21 - DNA, 35 bp, Artificial Sequence
  primer
ggagatatacatatgccatttactgtcccaatctt

SEQ ID NO: 22 - DNA, 15 bp, Artificial Sequence
  primer
ttcatccatctgcag

SEQ ID NO: 23 - DNA, 15 bp, Artificial Sequence
  primer
ggagatatacatatg

SEQ ID NO: 24 - DNA, 35 bp, Artificial Sequence
  primer
ttcatccatctgcaggagcacccattgttggggtt

SEQ ID NO: 25 - DNA, 35 bp, Artificial Sequence
  primer
ggagatatacatatgctgtctcctgtcaacatctg

SEQ ID NO: 26 - DNA, 35 bp, Artificial Sequence
  primer
ttcatccatctgcagttgcttgagtgttcggcctg

SEQ ID NO: 27 - DNA, 35 bp, Artificial Sequence
  primer
ggagatatacatatgattgagaggactatctatcg

SEQ ID NO: 28 - DNA, 36 bp, Artificial Sequence
  primer
ttcatccatctgcagcacatcctgaaaaccataaac

SEQ ID NO: 29 - DNA, 35 bp, Artificial Sequence
  primer
ggagatatacatatggtctctgggtcctgggtttc